European Patent Application EP 4 726 392 A1, published April 15, 2026. Title: Blood test for predicting sports-associated injuries. Applicant: UNIVERSITÄTSKLINIKUM KNAPPSCHAFTSKRANKENHAUS BOCHUM GMBH. The sequence listing filed with the application follows.

SEQUENCE LISTING (24 sequences)

SEQ ID NO: 1 - DNA, 738 bp, Homo sapiens
  source 1..738: mol_type = genomic DNA; note = Immature TFAM coding sequence, isoform 1
atggcgtttctccgaagcatgtggggcgtgctgagtgccctgggaaggtctggagcagagctgtgcaccggctgtggaagtcgactgcgctcccccttcagttttgtgtatttaccgaggtggttttcatctgtcttggcaagttgtccaaagaaacctgtaagttcttaccttcgattttctaaagaacaactacccatatttaaagctcagaacccagatgcaaaaactacagaactaattagaagaattgcccagcgttggagggaacttcctgattcaaagaaaaaaatatatcaagatgcttatagggcggagtggcaggtatataaagaagagataagcagatttaaagaacagctaactccaagtcagattatgtctttggaaaaagaaatcatggacaaacatttaaaaaggaaagctatgacaaaaaaaaaagagttaacactgcttggaaaaccaaaaagacctcgttcagcttataacgtttatgtagctgaaagattccaagaagctaagggtgattcaccgcaggaaaagctgaagactgtaaaggaaaactggaaaaatctgtctgactctgaaaaggaattatatattcagcatgctaaagaggacgaaactcgttatcataatgaaatgaagtcttgggaagaacaaatgattgaagttggacgaaaggatcttctacgtcgcacaataaagaaacaacgaaaatatggtgctgaggagtgt

SEQ ID NO: 2 - protein, 246 aa, Homo sapiens
  source 1..246: note = Immature TFAM coding sequence, isoform 1
MAFLRSMWGVLSALGRSGAELCTGCGSRLRSPFSFVYLPRWFSSVLASCPKKPVSSYLRFSKEQLPIFKAQNPDAKTTELIRRIAQRWRELPDSKKKIYQDAYRAEWQVYKEEISRFKEQLTPSQIMSLEKEIMDKHLKRKAMTKKKELTLLGKPKRPRSAYNVYVAERFQEAKGDSPQEKLKTVKENWKNLSDSEKELYIQHAKEDETRYHNEMKSWEEQMIEVGRKDLLRRTIKKQRKYGAEEC

SEQ ID NO: 3 - DNA, 612 bp, Homo sapiens
  source 1..612: mol_type = genomic DNA; note = Mature TFAM coding sequence, isoform 1
tcatctgtcttggcaagttgtccaaagaaacctgtaagttcttaccttcgattttctaaagaacaactacccatatttaaagctcagaacccagatgcaaaaactacagaactaattagaagaattgcccagcgttggagggaacttcctgattcaaagaaaaaaatatatcaagatgcttatagggcggagtggcaggtatataaagaagagataagcagatttaaagaacagctaactccaagtcagattatgtctttggaaaaagaaatcatggacaaacatttaaaaaggaaagctatgacaaaaaaaaaagagttaacactgcttggaaaaccaaaaagacctcgttcagcttataacgtttatgtagctgaaagattccaagaagctaagggtgattcaccgcaggaaaagctgaagactgtaaaggaaaactggaaaaatctgtctgactctgaaaaggaattatatattcagcatgctaaagaggacgaaactcgttatcataatgaaatgaagtcttgggaagaacaaatgattgaagttggacgaaaggatcttctacgtcgcacaataaagaaacaacgaaaatatggtgctgaggagtgt

SEQ ID NO: 4 - protein, 204 aa, Homo sapiens
  source 1..204: note = Mature TFAM coding sequence, isoform 1
SSVLASCPKKPVSSYLRFSKEQLPIFKAQNPDAKTTELIRRIAQRWRELPDSKKKIYQDAYRAEWQVYKEEISRFKEQLTPSQIMSLEKEIMDKHLKRKAMTKKKELTLLGKPKRPRSAYNVYVAERFQEAKGDSPQEKLKTVKENWKNLSDSEKELYIQHAKEDETRYHNEMKSWEEQMIEVGRKDLLRRTIKKQRKYGAEEC

SEQ ID NO: 5 - DNA, 642 bp, Homo sapiens
  source 1..642: mol_type = genomic DNA; note = Immature TFAM coding sequence, isoform 2
atggcgtttctccgaagcatgtggggcgtgctgagtgccctgggaaggtctggagcagagctgtgcaccggctgtggaagtcgactgcgctcccccttcagttttgtgtatttaccgaggtggttttcatctgtcttggcaagttgtccaaagaaacctgtaagttcttaccttcgattttctaaagaacaactacccatatttaaagctcagaacccagatgcaaaaactacagaactaattagaagaattgcccagcgttggagggaacttcctgattcaaagaaaaaaatatatcaagatgcttatagggcggagtggcaggtatataaagaagagataagcagatttaaagaacagctaactccaagtcagattatgtctttggaaaaagaaatcatggacaaacatttaaaaaggaaagctatgacaaaaaaaaaagaaaagctgaagactgtaaaggaaaactggaaaaatctgtctgactctgaaaaggaattatatattcagcatgctaaagaggacgaaactcgttatcataatgaaatgaagtcttgggaagaacaaatgattgaagttggacgaaaggatcttctacgtcgcacaataaagaaacaacgaaaatatggtgctgaggagtgt

SEQ ID NO: 6 - protein, 214 aa, Homo sapiens
  source 1..214: note = Immature TFAM protein, isoform 2
MAFLRSMWGVLSALGRSGAELCTGCGSRLRSPFSFVYLPRWFSSVLASCPKKPVSSYLRFSKEQLPIFKAQNPDAKTTELIRRIAQRWRELPDSKKKIYQDAYRAEWQVYKEEISRFKEQLTPSQIMSLEKEIMDKHLKRKAMTKKKEKLKTVKENWKNLSDSEKELYIQHAKEDETRYHNEMKSWEEQMIEVGRKDLLRRTIKKQRKYGAEEC

SEQ ID NO: 7 - DNA, 516 bp, Homo sapiens
  source 1..516: mol_type = genomic DNA; note = Mature TFAM coding sequence, isoform 2
tcatctgtcttggcaagttgtccaaagaaacctgtaagttcttaccttcgattttctaaagaacaactacccatatttaaagctcagaacccagatgcaaaaactacagaactaattagaagaattgcccagcgttggagggaacttcctgattcaaagaaaaaaatatatcaagatgcttatagggcggagtggcaggtatataaagaagagataagcagatttaaagaacagctaactccaagtcagattatgtctttggaaaaagaaatcatggacaaacatttaaaaaggaaagctatgacaaaaaaaaaagaaaagctgaagactgtaaaggaaaactggaaaaatctgtctgactctgaaaaggaattatatattcagcatgctaaagaggacgaaactcgttatcataatgaaatgaagtcttgggaagaacaaatgattgaagttggacgaaaggatcttctacgtcgcacaataaagaaacaacgaaaatatggtgctgaggagtgt

SEQ ID NO: 8 - protein, 172 aa, Homo sapiens
  source 1..172: note = Mature TFAM protein, isoform 2
SSVLASCPKKPVSSYLRFSKEQLPIFKAQNPDAKTTELIRRIAQRWRELPDSKKKIYQDAYRAEWQVYKEEISRFKEQLTPSQIMSLEKEIMDKHLKRKAMTKKKEKLKTVKENWKNLSDSEKELYIQHAKEDETRYHNEMKSWEEQMIEVGRKDLLRRTIKKQRKYGAEEC

SEQ ID NO: 9 - DNA, 1188 bp, Homo sapiens
  source 1..1188: mol_type = genomic DNA; note = Immature TFB2M coding sequence, isoform 1
atgtggatcccagtggtcgggcttcctcggcggctgaggctctccgccttggcgggcgctggtcgcttttgcattttagggtctgaagcggcgacgcgaaagcatttgccggcgaggaaccactgtgggctctctgactcctctccgcagctgtggcccgaaccggatttcaggaatccgccaaggaaggcgtctaaggccagcttagactttaagcgttacgtaaccgatcggagattggctgagaccctggcgcaaatctatttgggaaaaccaagtagacctccacacctactgctggagtgcaatccaggtcctggaatcctgactcaggcattacttgaagctggtgccaaagtggttgcgctcgaaagtgacaaaacttttattccacatttggagtccttaggaaaaaatctggatggaaaactacgagtgattcactgtgacttctttaaactagatcctagaagtggtggagtaataaaaccacctgctatgtcttctcgagggctctttaagaatttgggaatagaagcagttccttggacagcagacatccctttaaaagtagttggaatgttcccaagtagaggtgagaaaagggcactttggaaactcgcatatgacttgtattcctgtacttctatatataaatttggacgaatagaagtaaatatgtttattggtgaaaaagaattccagaaactaatggcagatcccggaaatccagacttgtatcatgtattaagtgttatctggcaattagcttgtgagattaaggttctgcacatggagccttggtcatcatttgatatatacacccggaaagggccgctggaaaacccaaagcgtagggaattattagaccaattacaacaaaagctgtatcttattcaaatgattcctcgtcaaaatttatttaccaagaacttaacacctatgaactataatatattttttcacttgttaaagcactgttttgggaggcgcagcgccactgtaatagaccacttacgttcattgactccacttgatgcgagagatatattgatgcaaataggaaaacaggaggatgagaaagtagttaacatgcaccctcaagacttcaaaacactttttgaaactatagagcgttccaaagattgtgcttataaatggctgtatgatgaaaccctggaagatagg

SEQ ID NO: 10 - protein, 396 aa, Homo sapiens
  source 1..396: note = Immature TFB2M coding sequence, isoform 1
MWIPVVGLPRRLRLSALAGAGRFCILGSEAATRKHLPARNHCGLSDSSPQLWPEPDFRNPPRKASKASLDFKRYVTDRRLAETLAQIYLGKPSRPPHLLLECNPGPGILTQALLEAGAKVVALESDKTFIPHLESLGKNLDGKLRVIHCDFFKLDPRSGGVIKPPAMSSRGLFKNLGIEAVPWTADIPLKVVGMFPSRGEKRALWKLAYDLYSCTSIYKFGRIEVNMFIGEKEFQKLMADPGNPDLYHVLSVIWQLACEIKVLHMEPWSSFDIYTRKGPLENPKRRELLDQLQQKLYLIQMIPRQNLFTKNLTPMNYNIFFHLLKHCFGRRSATVIDHLRSLTPLDARDILMQIGKQEDEKVVNMHPQDFKTLFETIERSKDCAYKWLYDETLEDR

SEQ ID NO: 11 - DNA, 1059 bp, Homo sapiens
  source 1..1059: mol_type = genomic DNA; note = Mature TFB2M coding sequence, isoform 1
ctctctgactcctctccgcagctgtggcccgaaccggatttcaggaatccgccaaggaaggcgtctaaggccagcttagactttaagcgttacgtaaccgatcggagattggctgagaccctggcgcaaatctatttgggaaaaccaagtagacctccacacctactgctggagtgcaatccaggtcctggaatcctgactcaggcattacttgaagctggtgccaaagtggttgcgctcgaaagtgacaaaacttttattccacatttggagtccttaggaaaaaatctggatggaaaactacgagtgattcactgtgacttctttaaactagatcctagaagtggtggagtaataaaaccacctgctatgtcttctcgagggctctttaagaatttgggaatagaagcagttccttggacagcagacatccctttaaaagtagttggaatgttcccaagtagaggtgagaaaagggcactttggaaactcgcatatgacttgtattcctgtacttctatatataaatttggacgaatagaagtaaatatgtttattggtgaaaaagaattccagaaactaatggcagatcccggaaatccagacttgtatcatgtattaagtgttatctggcaattagcttgtgagattaaggttctgcacatggagccttggtcatcatttgatatatacacccggaaagggccgctggaaaacccaaagcgtagggaattattagaccaattacaacaaaagctgtatcttattcaaatgattcctcgtcaaaatttatttaccaagaacttaacacctatgaactataatatattttttcacttgttaaagcactgttttgggaggcgcagcgccactgtaatagaccacttacgttcattgactccacttgatgcgagagatatattgatgcaaataggaaaacaggaggatgagaaagtagttaacatgcaccctcaagacttcaaaacactttttgaaactatagagcgttccaaagattgtgcttataaatggctgtatgatgaaaccctggaagatagg

SEQ ID NO: 12 - protein, 353 aa, Homo sapiens
  source 1..353: note = Mature TFB2M protein, isoform 1
LSDSSPQLWPEPDFRNPPRKASKASLDFKRYVTDRRLAETLAQIYLGKPSRPPHLLLECNPGPGILTQALLEAGAKVVALESDKTFIPHLESLGKNLDGKLRVIHCDFFKLDPRSGGVIKPPAMSSRGLFKNLGIEAVPWTADIPLKVVGMFPSRGEKRALWKLAYDLYSCTSIYKFGRIEVNMFIGEKEFQKLMADPGNPDLYHVLSVIWQLACEIKVLHMEPWSSFDIYTRKGPLENPKRRELLDQLQQKLYLIQMIPRQNLFTKNLTPMNYNIFFHLLKHCFGRRSATVIDHLRSLTPLDARDILMQIGKQEDEKVVNMHPQDFKTLFETIERSKDCAYKWLYDETLEDR

SEQ ID NO: 13 - DNA, 885 bp, Homo sapiens
  source 1..885: mol_type = genomic DNA; note = Immature TFB2M coding sequence, isoform X1
atgtggatcccagtggtcgggcttcctcggcggctgaggctctccgccttggcgggcgctggtcgcttttgcattttagggtctgaagcggcgacgcgaaagcatttgccggcgaggaaccactgtgggctctctgactcctctccgcagctgtggcccgaaccggatttcaggaatccgccaaggaaggcgtctaaggccagcttagactttaagcgttacgtaaccgatcggagattggctgagaccctggcgcaaatctatttgggaaaaccaagtagacctccacacctactgctggagtgcaatccaggtcctggaatcctgactcaggcattacttgaagctggtgccaaagtggttgcgctcgaaagtgacaaaacttttattccacatttggagaaactaatggcagatcccggaaatccagacttgtatcatgtattaagtgttatctggcaattagcttgtgagattaaggttctgcacatggagccttggtcatcatttgatatatacacccggaaagggccgctggaaaacccaaagcgtagggaattattagaccaattacaacaaaagctgtatcttattcaaatgattcctcgtcaaaatttatttaccaagaacttaacacctatgaactataatatattttttcacttgttaaagcactgttttgggaggcgcagcgccactgtaatagaccacttacgttcattgactccacttgatgcgagagatatattgatgcaaataggaaaacaggaggatgagaaagtagttaacatgcaccctcaagacttcaaaacactttttgaaactatagagcgttccaaagattgtgcttataaatggctgtatgatgaaaccctggaagatagg

SEQ ID NO: 14 - protein, 295 aa, Homo sapiens
  source 1..295: note = Immature TFB2M coding sequence, isoform X1
MWIPVVGLPRRLRLSALAGAGRFCILGSEAATRKHLPARNHCGLSDSSPQLWPEPDFRNPPRKASKASLDFKRYVTDRRLAETLAQIYLGKPSRPPHLLLECNPGPGILTQALLEAGAKVVALESDKTFIPHLEKLMADPGNPDLYHVLSVIWQLACEIKVLHMEPWSSFDIYTRKGPLENPKRRELLDQLQQKLYLIQMIPRQNLFTKNLTPMNYNIFFHLLKHCFGRRSATVIDHLRSLTPLDARDILMQIGKQEDEKVVNMHPQDFKTLFETIERSKDCAYKWLYDETLEDR

SEQ ID NO: 15 - DNA, 756 bp, Homo sapiens
  source 1..756: mol_type = genomic DNA; note = Mature TFB2M coding sequence, isoform X1
ctctctgactcctctccgcagctgtggcccgaaccggatttcaggaatccgccaaggaaggcgtctaaggccagcttagactttaagcgttacgtaaccgatcggagattggctgagaccctggcgcaaatctatttgggaaaaccaagtagacctccacacctactgctggagtgcaatccaggtcctggaatcctgactcaggcattacttgaagctggtgccaaagtggttgcgctcgaaagtgacaaaacttttattccacatttggagaaactaatggcagatcccggaaatccagacttgtatcatgtattaagtgttatctggcaattagcttgtgagattaaggttctgcacatggagccttggtcatcatttgatatatacacccggaaagggccgctggaaaacccaaagcgtagggaattattagaccaattacaacaaaagctgtatcttattcaaatgattcctcgtcaaaatttatttaccaagaacttaacacctatgaactataatatattttttcacttgttaaagcactgttttgggaggcgcagcgccactgtaatagaccacttacgttcattgactccacttgatgcgagagatatattgatgcaaataggaaaacaggaggatgagaaagtagttaacatgcaccctcaagacttcaaaacactttttgaaactatagagcgttccaaagattgtgcttataaatggctgtatgatgaaaccctggaagatagg

SEQ ID NO: 16 - protein, 252 aa, Homo sapiens
  source 1..252: note = Mature TFB2M protein, isoform X1
LSDSSPQLWPEPDFRNPPRKASKASLDFKRYVTDRRLAETLAQIYLGKPSRPPHLLLECNPGPGILTQALLEAGAKVVALESDKTFIPHLEKLMADPGNPDLYHVLSVIWQLACEIKVLHMEPWSSFDIYTRKGPLENPKRRELLDQLQQKLYLIQMIPRQNLFTKNLTPMNYNIFFHLLKHCFGRRSATVIDHLRSLTPLDARDILMQIGKQEDEKVVNMHPQDFKTLFETIERSKDCAYKWLYDETLEDR

SEQ ID NO: 17 - DNA, 609 bp, Homo sapiens
  source 1..609: mol_type = genomic DNA; note = Immature TFB2M coding sequence, isoform X2
atgttcccaagtagaggtgagaaaagggcactttggaaactcgcatatgacttgtattcctgtacttctatatataaatttggacgaatagaagtaaatatgtttattggtgaaaaagaattccagaaactaatggcagatcccggaaatccagacttgtatcatgtattaagtgttatctggcaattagcttgtgagattaaggttctgcacatggagccttggtcatcatttgatatatacacccggaaagggccgctggaaaacccaaagcgtagggaattattagaccaattacaacaaaagctgtatcttattcaaatgattcctcgtcaaaatttatttaccaagaacttaacacctatgaactataatatattttttcacttgttaaagcactgttttgggaggcgcagcgccactgtaatagaccacttacgttcattgactccacttgatgcgagagatatattgatgcaaataggaaaacaggaggatgagaaagtagttaacatgcaccctcaagacttcaaaacactttttgaaactatagagcgttccaaagattgtgcttataaatggctgtatgatgaaaccctggaagatagg

SEQ ID NO: 18 - protein, 203 aa, Homo sapiens
  source 1..203: note = Immature TFB2M protein, isoform X2
MFPSRGEKRALWKLAYDLYSCTSIYKFGRIEVNMFIGEKEFQKLMADPGNPDLYHVLSVIWQLACEIKVLHMEPWSSFDIYTRKGPLENPKRRELLDQLQQKLYLIQMIPRQNLFTKNLTPMNYNIFFHLLKHCFGRRSATVIDHLRSLTPLDARDILMQIGKQEDEKVVNMHPQDFKTLFETIERSKDCAYKWLYDETLEDR

SEQ ID NO: 19 - DNA, 18 bp, Homo sapiens
  source 1..18: mol_type = genomic DNA; note = TFAM and TFB2M consensus binding sequence 1
aaagataaaatttgaaat

SEQ ID NO: 20 - DNA, 17 bp, Homo sapiens
  source 1..17: mol_type = genomic DNA; note = TFAM and TFB2M consensus binding sequence 2
aaagacaccccccacag

SEQ ID NO: 21 - DNA, 126 bp, Homo sapiens
  source 1..126: mol_type = genomic DNA; note = N-terminal part of immature TFAM coding sequence
atggcgtttctccgaagcatgtggggcgtgctgagtgccctgggaaggtctggagcagagctgtgcaccggctgtggaagtcgactgcgctcccccttcagttttgtgtatttaccgaggtggttt

SEQ ID NO: 22 - protein, 42 aa, Homo sapiens
  source 1..42: note = N-terminal part of immature TFAM protein
MAFLRSMWGVLSALGRSGAELCTGCGSRLRSPFSFVYLPRWF

SEQ ID NO: 23 - DNA, 129 bp, Homo sapiens
  source 1..129: mol_type = genomic DNA; note = N-terminal part of immature TFB2M coding sequence
atgtggatcccagtggtcgggcttcctcggcggctgaggctctccgccttggcgggcgctggtcgcttttgcattttagggtctgaagcggcgacgcgaaagcatttgccggcgaggaaccactgtggg

SEQ ID NO: 24 - protein, 43 aa, Homo sapiens
  source 1..43: note = N-terminal part of immature TFB2M protein
MWIPVVGLPRRLRLSALAGAGRFCILGSEAATRKHLPARNHCG